European Patent Specification EP 3 305 321 B1, published October 16, 2024. Title: Medicament and method for treating pulmonary hypertension. Applicant: University of Toyama Kyowa Hakko Kirin, Co., LTD. The sequence listing filed with the application follows.

SEQUENCE LISTING (34 sequences)

SEQ ID NO: 1 - protein, 5 aa, Artificial Sequence
  HCDR1
SYVIH

SEQ ID NO: 2 - protein, 17 aa, Artificial Sequence
  HCDR2
YINPYNDGTKYNERFKG

SEQ ID NO: 3 - protein, 12 aa, Artificial Sequence
  HCDR3
EGIRYYGLLGDY

SEQ ID NO: 4 - protein, 11 aa, Artificial Sequence
  LCDR1
GTSEDIINYLN

SEQ ID NO: 5 - protein, 7 aa, Artificial Sequence
  LCDR2
HTSRLQS

SEQ ID NO: 6 - protein, 9 aa, Artificial Sequence
  LCDR3
QQGYTLPYT

SEQ ID NO: 7 - protein, 121 aa, Artificial Sequence [sequence omitted]

SEQ ID NO: 8 - protein, 107 aa, Artificial Sequence [sequence omitted]

SEQ ID NO: 9 - protein, 451 aa, Artificial Sequence
  Benralizumab heavy chain
EVQLVQSGAEVKKPGASVKVSCKASGYTFTSYVIHWVRQRPGQGLAWMGYINPYNDGTKYNERFKGKVTITSDRSTSTVYMELSSLRSEDTAVYLCGREGIRYYGLLGDYWGQGTLVTVSSASTKGPSVFPLAPSSKSTSGGTAALGCLVKDYFPEPVTVSWNSGALTSGVHTFPAVLQSSGLYSLSSVVTVPSSSLGTQTYICNVNHKPSNTKVDKKVEPKSCDKTHTCPPCPAPELLGGPSVFLFPPKPKDTLMISRTPEVTCVVVDVSHEDPEVKFNWYVDGVEVHNAKTKPREEQYNSTYRVVSVLTVLHQDWLNGKEYKCKVSNKALPAPIEKTISKAKGQPREPQVYTLPPSRDELTKNQVSLTCLVKGFYPSDIAVEWESNGQPENNYKTTPPVLDSDGSFFLYSKLTVDKSRWQQGNVFSCSVMHEALHNHYTQKSLSLSPGK

SEQ ID NO: 10 - protein, 155 aa, Artificial Sequence
  Benralizumab light chain
DIQMTQSPSSLSASVGDRVTITCGTSEDIINYLNWYQQKPGKAPKLLIYHTSRLQSGVPSRFSGSGSGTDFTLTISSLQPEDFATYYCQQGYTLPYTFGQGTKVEIKRTVAAPSVFIFPPSDEQLKSGTASVVCLLNNFYPREAKVQWKVDNALQ

SEQ ID NO: 11 - DNA, 21 bp, Artificial Sequence
  rat kappa re
gccatcaatgttccacttgac

SEQ ID NO: 12 - DNA, 22 bp, Artificial Sequence
  rat gamma re
gtkacyggctcagggaaatagc

SEQ ID NO: 13 - DNA, 381 bp, Artificial Sequence
  H7 VL DNA with signal sequence
atgggtgtccccactcagctcctggggttgttgctactgtggattacagatgccatatgtgacatccagatgacacagtctccagcttccctgtctgcatctctgggagaaactgtcaccatcgaatgtcgaacaagtgaggacatttacaatggtttagcatggtatcagcagaagccagggaaatctcctcagctcctgatctataatgcaaatagtttgcatactggggtcccatcacggttcagtggcagtggatctggtacacagtattctctcaagataaacagtctgcaatctgaagatgtcgcaagttattgctgtcaacagtattccaattatcctttcacgttcggctcagggacgaagttggaaataaaa

SEQ ID NO: 14 - protein, 127 aa, Artificial Sequence
  H7 VL AA with signal sequence
MGVPTQLLGLLLLWITDAICDIQMTQSPASLSASLGETVTIECRTSEDIYNGLAWYQQKPGKSPQLLIYNANSLHTGVPSRFSGSGSGTQYSLKINSLQSEDVASYCCQQYSNYPFTFGSGTKLEIK

SEQ ID NO: 15 - protein, 107 aa, Artificial Sequence
  H7 VL AA without signal sequence
DIQMTQSPASLSASLGETVTIECRTSEDIYNGLAWYQQKPGKSPQLLIYNANSLHTGVPSRFSGSGSGTQYSLKINSLQSEDVASYCCQQYSNYPFTFGSGTKLEIK

SEQ ID NO: 16 - DNA, 429 bp, Artificial Sequence
  H7 VH DNA with signal sequence
atgaaatgcagctggatcatcctcttcttgatggcactaactacaggggtcaactcagaagtccagctgcagcagtctggggctgagcttgggaaacctgggacctcagtcaagttgtcttgcaaggtttctggctataacattaagaatacctacatacactgggtgaatcagaggcctggaaagggcctggaatggataggaaggattgatcctgcaaatggaaatcctatatatgctgagaagttcaaaaacaaggccacactgactgcagatacatcgtccaacacagcctacatgcaactcagccaactgaaatctgacgacacagcaatctatttttgtgctatgcatcgggggcatagtatgggtcccggcccgtatgttatggatgcctggggtcaaggagcttcagtcactgtctcctca

SEQ ID NO: 17 - protein, 143 aa, Artificial Sequence
  H7 VH AA with signal sequence
MKCSWIILFLMALTTGVNSEVQLQQSGAELGKPGTSVKLSCKVSGYNIKNTYIHWVNQRPGKGLEWIGRIDPANGNPIYAEKFKNKATLTADTSSNTAYMQLSQLKSDDTAIYFCAMHRGHSMGPGPYVMDAWGQGASVTVSS

SEQ ID NO: 18 - protein, 124 aa, Artificial Sequence
  H7 VH AA without signal sequence
EVQLQQSGAELGKPGTSVKLSCKVSGYNIKNTYIHWVNQRPGKGLEWIGRIDPANGNPIYAEKFKNKATLTADTSSNTAYMQLSQLKSDDTAIYFCAMHRGHSMGPGPYVMDAWGQGASVTVSS

SEQ ID NO: 19 - DNA, 45 bp, Artificial Sequence
  VL fw
tcccgcgtcctctagtgacatccagatgacacagtctccagcttc

SEQ ID NO: 20 - DNA, 44 bp, Artificial Sequence
  VL re
gtgcagccaccgtacgttttatttccaacttcgtccctgagccg

SEQ ID NO: 21 - DNA, 45 bp, Artificial Sequence
  VH fw
aagggcgtgcagtgcgaagtccagctgcagcagtctggggctgag

SEQ ID NO: 22 - DNA, 45 bp, Artificial Sequence
  VH re
ggcccttggtgctagctgaggagacagtgactgaagctccttgac

SEQ ID NO: 23 - DNA, 31 bp, Artificial Sequence
  VL(CS) fw
agttattcctgtcaacagtattccaattatc

SEQ ID NO: 24 - DNA, 29 bp, Artificial Sequence
  VL(CS) re
ttgacaggaataacttgcgacatcttcag

SEQ ID NO: 25 - DNA, 381 bp, Artificial Sequence; identical to SEQ ID NO: 13
  H7 VL DNA for recombinant expression

SEQ ID NO: 26 - DNA, 381 bp, Artificial Sequence
  H7(CS) VL DNA for recombinant expression
atgggtgtccccactcagctcctggggttgttgctactgtggattacagatgccatatgtgacatccagatgacacagtctccagcttccctgtctgcatctctgggagaaactgtcaccatcgaatgtcgaacaagtgaggacatttacaatggtttagcatggtatcagcagaagccagggaaatctcctcagctcctgatctataatgcaaatagtttgcatactggggtcccatcacggttcagtggcagtggatctggtacacagtattctctcaagataaacagtctgcaatctgaagatgtcgcaagttattcctgtcaacagtattccaattatcctttcacgttcggctcagggacgaagttggaaataaaa

SEQ ID NO: 27 - DNA, 429 bp, Artificial Sequence; identical to SEQ ID NO: 16
  H7 or H7(CS) hIgG1 VH DNA for recombinant expression

SEQ ID NO: 28 - DNA, 429 bp, Artificial Sequence; identical to SEQ ID NO: 16
  H7 or H7(CS) hIgG1(N297A) VH DNA for recombinant expression

SEQ ID NO: 29 - DNA, 396 bp, Artificial Sequence
  rtDNP-1 VL DNA with signal sequence
atgaatctgcccgtgcatctgctggtgctgctgctgttctggatccccgcctcccgcggggatgtggtgatgactcagactcccgtgtccctgcccgtgtccctgggggggcaggcctccatctcctgtcgctcctcccagtccctggccaattcctatgggaatacttatctgtcctggtatctgcagaagcccgggcagtccccccagctgctgatctatcgcgtgtccaatactttctccggggtgcccgatcgcttctccgggtccgggtccgggactgatttcactctgaagatctcccgcgtggagcccgaggatctgggggattattattgtctgcaggggactcatcagccctatactttcggggccgggactaagctggagctgaag

SEQ ID NO: 30 - protein, 132 aa, Artificial Sequence
  rtDNP-1 VL AA with signal sequence
MNLPVHLLVLLLFWIPASRGDVVMTQTPVSLPVSLGGQASISCRSSQSLANSYGNTYLSWYLQKPGQSPQLLIYRVSNTFSGVPDRFSGSGSGTDFTLKISRVEPEDLGDYYCLQGTHQPYTFGAGTKLELK

SEQ ID NO: 31 - protein, 112 aa, Artificial Sequence
  rtDNP-1 VL AA without signal sequence
DVVMTQTPVSLPVSLGGQASISCRSSQSLANSYGNTYLSWYLQKPGQSPQLLIYRVSNTFSGVPDRFSGSGSGTDFTLKISRVEPEDLGDYYCLQGTHQPYTFGAGTKLELK

SEQ ID NO: 32 - DNA, 405 bp, Artificial Sequence
  rtDNP-1 VH DNA with signal sequence
atgatggtgctgtccctgctgtatctgctgactgccctgcccgggatcctgtccgaggtgcagctgcaggagtccgggcccgggctggtgaagccctcccagtccctgtccctgacttgttccgtgactgggtattccatcacttccgggtattggaattggatccgcaagttccccgggaataagatggagtggatcgggtatatctcctattccgggtccacttattataatccctccctgaagtcccgcatctccatcactcgcgatacttccaagaatcagttcttcctgcagctgaattccgtgactactgaggatactgccacttattattgtgcccgctggggggtgcgccattatttcgattattgggggcagggggtgatggccactgtgtcctcc

SEQ ID NO: 33 - protein, 135 aa, Artificial Sequence
  rtDNP-1 VH AA with signal sequence
MMVLSLLYLLTALPGILSEVQLQESGPGLVKPSQSLSLTCSVTGYSITSGYWNWIRKFPGNKMEWIGYISYSGSTYYNPSLKSRISITRDTSKNQFFLQLNSVTTEDTATYYCARWGVRHYFDYWGQGVMATVSS

SEQ ID NO: 34 - protein, 117 aa, Artificial Sequence
  rtDNP-1 VH AA without signal sequence
EVQLQESGPGLVKPSQSLSLTCSVTGYSITSGYWNWIRKFPGNKMEWIGYISYSGSTYYNPSLKSRISITRDTSKNQFFLQLNSVTTEDTATYYCARWGVRHYFDYWGQGVMATVSS